European Patent Specification EP 3 481 420 B1, published August 13, 2025. Title: ANTIBODY FORMULATIONS. Applicant: SANOFI. The sequence listing filed with the application follows.

SEQUENCE LISTING (69 sequences)

SEQ ID NO: 1 - protein, 36 aa, Homo sapiens
MNYPTLEMDLENLEDLFWELDRLDNYNTSLVENHLC

SEQ ID NO: 2 - DNA, 32 bp, Artificial Sequence
  Description of Artificial Sequence: Synthetic primer
  misc_feature (18)..(18): n is a, c, g, or t
cttccggaattcsargtnmagctgsagsagtc

SEQ ID NO: 3 - DNA, 35 bp, Artificial Sequence
  Description of Artificial Sequence: Synthetic primer
  misc_feature (18)..(18): n is a, c, g, or t
cttccggaattcsargtnmagctgsagsagtcwgg

SEQ ID NO: 4 - DNA, 36 bp, Artificial Sequence
  Description of Artificial Sequence: Synthetic primer
ggaggatccatagacagatgggggtgtcgttttggc

SEQ ID NO: 5 - DNA, 31 bp, Artificial Sequence
  Description of Artificial Sequence: Synthetic primer
ggagctcgayattgtgmtsacmcarwctmca

SEQ ID NO: 6 - DNA, 46 bp, Artificial Sequence
  Description of Artificial Sequence: Synthetic primer
tatagagctcaagcttggatggtgggaagatggatacagttggtgc

SEQ ID NO: 7 - DNA, 18 bp, Artificial Sequence
  Description of Artificial Sequence: Synthetic primer
ccaagctgtgtcctrtcc

SEQ ID NO: 8 - DNA, 32 bp, Artificial Sequence
  Description of Artificial Sequence: Synthetic primer
cgacaagtcgactagcccttgaccaggcatcc

SEQ ID NO: 9 - DNA, 18 bp, Artificial Sequence
  Description of Artificial Sequence: Synthetic primer
wtctctrgagtcagtggg

SEQ ID NO: 10 - DNA, 32 bp, Artificial Sequence
  Description of Artificial Sequence: Synthetic primer
cgactagtcgactggtgggaagatggatacag

SEQ ID NO: 11 - protein, 112 aa, Mus sp.
DIVMTQAAPSVAVTPRESVSISCRSSKSLLHSSGKTYLYWFLQRPGQSPQLLIYRMSNLASGVPDRFSGSGSGTAFTLRISRVEAEDVGVYYCMQHLEYPYTFGGGTKLEIK

SEQ ID NO: 12 - protein, 111 aa, Mus sp.
QVQLKESGPGLVAPSQSLSITCTVSGFSLIDYGVNWIRQPPGKGLEWLGVIWGDGTTYYNSALKSRLSIRKDNSQSQVFLKMNSLQTDDTAMYYCARIVYWGQGTLVTVSA

SEQ ID NO: 13 - protein, 112 aa, Artificial Sequence
  Description of Artificial Sequence: Synthetic polypeptide
DIVMTQSALSVAVTPGESVSISCRSSKSLLHSSGKTYLYWFLQRPGQSPQLLIYRMSNLASGVPDRFSGSGSGTAFTLKISRVEAEDVGVYYCMQHLEYPYTFGGGTKLEIK

SEQ ID NO: 14 - protein, 112 aa, Artificial Sequence
  Description of Artificial Sequence: Synthetic polypeptide
DIVMTQSALSVAVTPGESVSISCRSSKSLLHSSGKTYLYWFLQRPGQSPQLLIYRLSNLASGVPDRFSGSGSGTAFTLKISRVEAEDVGVYYCMQHLEYPYTFGGGTKLEIK

SEQ ID NO: 15 - protein, 113 aa, Artificial Sequence
  Description of Artificial Sequence: Synthetic polypeptide
DIVMTQSALSVAVTPGESVSISCRSSKSLLHSSGKTYLYWFLQRPGQSPQLLIYRLSSNLASGVPDRFSGSGSGTAFTLKISRVEAEDVGVYYCMQHLEYPYTFGGGTKLEIK

SEQ ID NO: 16 - protein, 111 aa, Artificial Sequence
  Description of Artificial Sequence: Synthetic polypeptide
QVQLQESGPGLVAPSESLSITCTVSGFSLIDYGVNWIRQPPGKGLEWLGVIWGDGTTYYNPSLKSRLSISKDNSKSQVFLKMNSLTAADTAMYYCARIVYWGQGTLVTVSS

SEQ ID NO: 17 - protein, 238 aa, Artificial Sequence
  Description of Artificial Sequence: Synthetic polypeptide
MGWSCIILFLVATATGVHSDIVMTQSALSVAVTPGESVSISCRSSKSLLHSSGKTYLYWFLQRPGQSPQLLIYRMSNLASGVPDRFSGSGSGTAFTLKISRVEAEDVGVYYCMQHLEYPYTFGGGTKLEIKRTVAAPSVFIFPPSDEQLKSGTASVVCLLNNFYPREAKVQWKVDNALQSGNSQESVTEQDSKDSTYSLSSTLTLSKADYEKHKVYACEVTHQGLSSPVTKSFNRGEC

SEQ ID NO: 18 - DNA, 731 bp, Artificial Sequence
  Description of Artificial Sequence: Synthetic polynucleotide
gctagcaccatgggctggagctgcatcatcctgttcctggtggccaccgccaccggcgtgcacagcgacatcgtgatgacccagagcgccctcagcgtggccgtgacccccggcgagagcgtgagcatcagctgccgcagcagcaagagcctgctgcacagcagcggcaagacctacctgtactggttcctgcagcgccccggccagagcccccagctgctgatctaccgcatgagcaacctggccagcggcgtgcccgaccgcttcagcggcagcggcagcggcaccgccttcaccctgaagatcagccgcgtggaggccgaggacgtgggcgtgtactactgcatgcagcacctggagtacccctacaccttcggcggcggcaccaagctggagatcaagcgtacggtggccgctccttccgtgttcatcttccctccctccgacgagcagctgaagtccggcaccgcctccgtggtgtgtctgctgaacaacttctaccctcgggaggccaaggtgcagtggaaggtggacaacgccctgcagtccggcaactcccaggagtccgtcaccgagcaggactccaaggacagcacctactccctgtcctccaccctgaccctgtccaaggccgactacgagaagcacaaggtgtacgcctgtgaggtgacccaccagggcctgtccagccctgtgaccaagtccttcaaccggggcgagtgctgaagctt

SEQ ID NO: 19 - protein, 238 aa, Artificial Sequence
  Description of Artificial Sequence: Synthetic polypeptide
MGWSCIILFLVATATGVHSDIVMTQSALSVAVTPGESVSISCRSSKSLLHSSGKTYLYWFLQRPGQSPQLLIYRLSNLASGVPDRFSGSGSGTAFTLKISRVEAEDVGVYYCMQHLEYPYTFGGGTKLEIKRTVAAPSVFIFPPSDEQLKSGTASVVCLLNNFYPREAKVQWKVDNALQSGNSQESVTEQDSKDSTYSLSSTLTLSKADYEKHKVYACEVTHQGLSSPVTKSFNRGEC

SEQ ID NO: 20 - DNA, 731 bp, Artificial Sequence
  Description of Artificial Sequence: Synthetic polynucleotide
gctagcaccatgggctggagctgcatcatcctgttcctggtggccaccgccaccggcgtgcacagcgacatcgtgatgacccagagcgccctcagcgtggccgtgacccccggcgagagcgtgagcatcagctgccgcagcagcaagagcctgctgcacagcagcggcaagacctacctgtactggttcctgcagcgccccggccagagcccccagctgctgatctaccgcctgagcaacctggccagcggcgtgcccgaccgcttcagcggcagcggcagcggcaccgccttcaccctgaagatcagccgcgtggaggccgaggacgtgggcgtgtactactgcatgcagcacctggagtacccctacaccttcggcggcggcaccaagctggagatcaagcgtacggtggccgctccttccgtgttcatcttccctccctccgacgagcagctgaagtccggcaccgcctccgtggtgtgtctgctgaacaacttctaccctcgggaggccaaggtgcagtggaaggtggacaacgccctgcagtccggcaactcccaggagtccgtcaccgagcaggactccaaggacagcacctactccctgtcctccaccctgaccctgtccaaggccgactacgagaagcacaaggtgtacgcctgtgaggtgacccaccagggcctgtccagccctgtgaccaagtccttcaaccggggcgagtgctgaagctt

SEQ ID NO: 21 - protein, 238 aa, Artificial Sequence
  Description of Artificial Sequence: Synthetic polypeptide
MGWSCIILFLVATATGVHSDIVMTQSALSVAVTPGESVSISCRSSKSLLHSSGKTYLYWFLQRPGQSPQLLIYRLSSLASGVPDRFSGSGSGTAFTLKISRVEAEDVGVYYCMQHLEYPYTFGGGTKLEIKRTVAAPSVFIFPPSDEQLKSGTASVVCLLNNFYPREAKVQWKVDNALQSGNSQESVTEQDSKDSTYSLSSTLTLSKADYEKHKVYACEVTHQGLSSPVTKSFNRGEC

SEQ ID NO: 22 - DNA, 731 bp, Artificial Sequence
  Description of Artificial Sequence: Synthetic polynucleotide
gctagcaccatgggctggagctgcatcatcctgttcctggtggccaccgccaccggcgtgcacagcgacatcgtgatgacccagagcgccctcagcgtggccgtgacccccggcgagagcgtgagcatcagctgccgcagcagcaagagcctgctgcacagcagcggcaagacctacctgtactggttcctgcagcgccccggccagagcccccagctgctgatctaccgcctgagcagcctggccagcggcgtgcccgaccgcttcagcggcagcggcagcggcaccgccttcaccctgaagatcagccgcgtggaggccgaggacgtgggcgtgtactactgcatgcagcacctggagtacccctacaccttcggcggcggcaccaagctggagatcaagcgtacggtggccgctccttccgtgttcatcttccctccctccgacgagcagctgaagtccggcaccgcctccgtggtgtgtctgctgaacaacttctaccctcgggaggccaaggtgcagtggaaggtggacaacgccctgcagtccggcaactcccaggagtccgtcaccgagcaggactccaaggacagcacctactccctgtcctccaccctgaccctgtccaaggccgactacgagaagcacaaggtgtacgcctgtgaggtgacccaccagggcctgtccagccctgtgaccaagtccttcaaccggggcgagtgctgaagctt

SEQ ID NO: 23 - protein, 456 aa, Artificial Sequence
  Description of Artificial Sequence: Synthetic polypeptide
MGWSCIILFLVATATGVHSQVQLQESGPGLVAPSESLSITCTVSGFSLIDYGVNWIRQPPGKGLEWLGVIWGDGTTYYNPSLKSRLSISKDNSKSQVFLKMNSLTAADTAMYYCARIVYWGQGTLVTVSSASTKGPSVFPLAPCSRSTSESTAALGCLVKDYFPEPVTVSWNSGALTSGVHTFPAVLQSSGLYSLSSVVTVPSSSLGTKTYTCNVDHKPSNTKVDKRVESKYGPPCPSCPAPEFLGGPSVFLFPPKPKDTLMISRTPEVTCVVVDVSQEDPEVQFNWYVDGVEVHNAKTKPREEQFNSTYRVVSVLTVLHQDWLNGKEYKCKVSNKGLPSSIEKTISKAKGQPREPQVYTLPPSQEEMTKNQVSLTCLVKGFYPSDIAVEWESNGQPENNYKTTPPVLDSDGSFFLYSRLTVDKSRWQEGNVFSCSVMHEALHNHYTQKSLSLSLG

SEQ ID NO: 24 - DNA, 1385 bp, Artificial Sequence
  Description of Artificial Sequence: Synthetic polynucleotide
gctagcaccatgggctggagctgcatcatcctgttcctggtggccaccgccaccggcgtgcacagccaggtgcagctgcaggagagcggccccggcctggtggcccccagcgagagcctgagcatcacctgcaccgtgagcggcttcagcctgatcgactacggcgtgaactggatccgccagccccccggcaagggcctggagtggctgggcgtgatctggggcgacggcaccacctactacaaccccagcctgaagagccgcctgagcatctccaaggacaacagcaagagccaggtgttcctgaagatgaacagcctgaccgccgccgacaccgccatgtactactgcgcccgcatcgtgtactggggccagggcaccctggtgaccgtgagcagcgccagcaccaagggcccttccgtgttccctctggccccttgctcccggtccacctccgagtccaccgccgctctgggctgcctggtgaaggactacttccctgagcctgtgaccgtgtcctggaactctggcgccctgacctccggcgtgcacaccttccctgccgtgctgcagtcctccggcctgtactccctgtcctccgtggtgaccgtgccttcctcctccctgggcaccaagacctacacctgtaacgtggaccacaagccttccaacaccaaggtggacaagcgggtggagtccaagtacggccctccttgcccttcctgccctgcccctgagttcctgggcggacctagcgtgttcctgttccctcctaagcctaaggacaccctgatgatctcccggacccctgaggtgacctgtgtggtggtggacgtgtcccaggaggaccctgaggtccagttcaactggtacgtggacggcgtggaggtgcacaacgccaagaccaagcctcgggaggagcagttcaattccacctaccgggtggtgtctgtgctgaccgtgctgcaccaggactggctgaacggcaaagaatacaagtgtaaggtctccaacaagggcctgccctcctccatcgagaaaaccatctccaaggccaagggccagcctagggagcctcaggtgtacaccctgcctcctagccaggaagagatgaccaagaaccaggtgtccctgacctgtctggtgaagggcttctacccttccgacatcgccgtggagtgggagtccaacggccagcctgagaacaactacaagaccacccctcctgtgctggactccgacggctccttcttcctgtactccaggctgaccgtggacaagtcccggtggcaggagggcaacgtcttttcctgctccgtgatgcacgaggccctgcacaaccactacacccagaagtccctgtccctgtctctgggctgaagctt

SEQ ID NO: 25 - protein, 22 aa, Homo sapiens
KPGQPPRLLIYDASNRATGIPA

SEQ ID NO: 26 - protein, 12 aa, Mus musculus
TDDTAMYYCARI

SEQ ID NO: 27 - protein, 12 aa, Homo sapiens
SEDSALYYCARD

SEQ ID NO: 28 - protein, 112 aa, Mus musculus; identical to SEQ ID NO: 11

SEQ ID NO: 29 - protein, 111 aa, Mus musculus; identical to SEQ ID NO: 12

SEQ ID NO: 30 - protein, 112 aa, Artificial Sequence
  Description of Artificial Sequence: Synthetic polypeptide
DIVMTQAAPSVAVTPGASVSISCRSSKSLLHSSGKTYLYWFLQRPGQSPQLLIYRMSNLASGVPDRFSGSGSGTAFTLRISRVEAEDVGVYYCMQHLEYPYTFGGGTKLEIK

SEQ ID NO: 31 - protein, 112 aa, Artificial Sequence
  Description of Artificial Sequence: Synthetic polypeptide
DIVMTQAAPSVAVTPGASVSISCRSSKSLLHSSGKTYLYWFLQRPGQSPQLLIYRLSNLASGVPDRFSGSGSGTAFTLRISRVEAEDVGVYYCMQHLEYPYTFGGGTKLEIK

SEQ ID NO: 32 - protein, 112 aa, Artificial Sequence
  Description of Artificial Sequence: Synthetic polypeptide
DIVMTQAAPSVAVTPGASVSISCRSSKSLLHSSGKTYLYWFLQRPGQSPQLLIYRLSSLASGVPDRFSGSGSGTAFTLRISRVEAEDVGVYYCMQHLEYPYTFGGGTKLEIK

SEQ ID NO: 33 - protein, 111 aa, Artificial Sequence
  Description of Artificial Sequence: Synthetic polypeptide
QVQLKESGPGLVAPSESLSITCTVSGFSLIDYGVNWIRQPPGKGLEWLGVIWGDGTTYYNPSLKSRLSISKDNSKSQVFLKVTSLTTDDTAMYYCARIVYWGQGTLVTVSA

SEQ ID NO: 34 - protein, 111 aa, Artificial Sequence
  Description of Artificial Sequence: Synthetic polypeptide
EVQLKESGPGLVAPGGSLSITCTVSGFSLIDYGVNWIRQPPGKGLEWLGVIWGDGTTYYNAPLKGRLSISKDNSKSQVFLQMNSLKTDDTAMYYCARIVYWGQGTLVTVSS

SEQ ID NO: 35 - protein, 238 aa, Artificial Sequence
  Description of Artificial Sequence: Synthetic polypeptide
MGWSCIILFLVATATGVHSDIVMTQAAPSVAVTPRESVSISCRSSKSLLHSSGKTYLYWFLQRPGQSPQLLIYRMSNLASGVPDRFSGSGSGTAFTLRISRVEAEDVGVYYCMQHLEYPYTFGGGTKLEIKRTVAAPSVFIFPPSDEQLKSGTASVVCLLNNFYPREAKVQWKVDNALQSGNSQESVTEQDSKDSTYSLSSTLTLSKADYEKHKVYACEVTHQGLSSPVTKSFNRGEC

SEQ ID NO: 36 - DNA, 731 bp, Artificial Sequence
  Description of Artificial Sequence: Synthetic polynucleotide
gctagcaccatgggctggagctgcatcatcctgttcctggtggccaccgccaccggcgtgcacagcgacatcgtgatgacccaggccgcccccagcgtggccgtgaccccccgcgagagcgtgagcatcagctgccgcagcagcaagagcctgctgcacagcagcggcaagacctacctgtactggttcctgcagcgccccggccagagcccccagctgctgatctaccgcatgagcaacctggccagcggcgtgcccgaccgcttcagcggcagcggcagcggcaccgccttcaccctgcgcatcagccgcgtggaggccgaggacgtgggcgtgtactactgcatgcagcacctggagtacccctacaccttcggcggcggcaccaagctggagatcaagcgtacggtggccgctccttccgtgttcatcttccctccctccgacgagcagctgaagtccggcaccgcctccgtggtgtgtctgctgaacaacttctaccctcgggaggccaaggtgcagtggaaggtggacaacgccctgcagtccggcaactcccaggagtccgtcaccgagcaggactccaaggacagcacctactccctgtcctccaccctgaccctgtccaaggccgactacgagaagcacaaggtgtacgcctgtgaggtgacccaccagggcctgtccagccctgtgaccaagtccttcaaccggggcgagtgctgaagctt

SEQ ID NO: 37 - protein, 456 aa, Artificial Sequence
  Description of Artificial Sequence: Synthetic polypeptide
MGWSCIILFLVATATGVHSQVQLKESGPGLVAPSQSLSITCTVSGFSLIDYGVNWIRQPPGKGLEWLGVIWGDGTTYYNSALKSRLSIRKDNSQSQVFLKMNSLQTDDTAMYYCARIVYWGQGTLVTVSAASTKGPSVFPLAPCSRSTSESTAALGCLVKDYFPEPVTVSWNSGALTSGVHTFPAVLQSSGLYSLSSVVTVPSSSLGTKTYTCNVDHKPSNTKVDKRVESKYGPPCPSCPAPEFLGGPSVFLFPPKPKDTLMISRTPEVTCVVVDVSQEDPEVQFNWYVDGVEVHNAKTKPREEQFNSTYRVVSVLTVLHQDWLNGKEYKCKVSNKGLPSSIEKTISKAKGQPREPQVYTLPPSQEEMTKNQVSLTCLVKGFYPSDIAVEWESNGQPENNYKTTPPVLDSDGSFFLYSRLTVDKSRWQEGNVFSCSVMHEALHNHYTQKSLSLSLG

SEQ ID NO: 38 - DNA, 1385 bp, Artificial Sequence
  Description of Artificial Sequence: Synthetic polynucleotide
gctagcaccatgggctggagctgcatcatcctgttcctggtggccaccgccaccggcgtgcacagccaggtgcagctgaaggagagcggccccggcctggtggcccccagccagagcctgagcatcacctgcaccgtgagcggcttcagcctgatcgactacggcgtgaactggatccgccagccccccggcaagggcctggagtggctgggcgtgatctggggcgacggcaccacctactacaacagcgccctgaagagccgcctgagcatccgcaaggacaacagccagagccaggtgttcctgaagatgaacagcctgcagaccgacgacaccgccatgtactactgcgcccgcatcgtgtactggggccagggcaccctggtgaccgtgagcgccgccagcaccaagggcccttccgtgttccctctggccccttgctcccggtccacctccgagtccaccgccgctctgggctgcctggtgaaggactacttccctgagcctgtgaccgtgtcctggaactctggcgccctgacctccggcgtgcacaccttccctgccgtgctgcagtcctccggcctgtactccctgtcctccgtggtgaccgtgccttcctcctccctgggcaccaagacctacacctgtaacgtggaccacaagccttccaacaccaaggtggacaagcgggtggagtccaagtacggccctccttgcccttcctgccctgcccctgagttcctgggcggacctagcgtgttcctgttccctcctaagcctaaggacaccctgatgatctcccggacccctgaggtgacctgtgtggtggtggacgtgtcccaggaggaccctgaggtccagttcaactggtacgtggacggcgtggaggtgcacaacgccaagaccaagcctcgggaggagcagttcaattccacctaccgggtggtgtctgtgctgaccgtgctgcaccaggactggctgaacggcaaagaatacaagtgtaaggtctccaacaagggcctgccctcctccatcgagaaaaccatctccaaggccaagggccagcctagggagcctcaggtgtacaccctgcctcctagccaggaagagatgaccaagaaccaggtgtccctgacctgtctggtgaagggcttctacccttccgacatcgccgtggagtgggagtccaacggccagcctgagaacaactacaagaccacccctcctgtgctggactccgacggctccttcttcctgtactccaggctgaccgtggacaagtcccggtggcaggagggcaacgtcttttcctgctccgtgatgcacgaggccctgcacaaccactacacccagaagtccctgtccctgtctctgggctgaagctt

SEQ ID NO: 39 - protein, 238 aa, Artificial Sequence
  Description of Artificial Sequence: Synthetic polypeptide
MGWSCIILFLVATATGVHSDIVMTQAAPSVAVTPGASVSISCRSSKSLLHSSGKTYLYWFLQRPGQSPQLLIYRMSNLASGVPDRFSGSGSGTAFTLRISRVEAEDVGVYYCMQHLEYPYTFGGGTKLEIKRTVAAPSVFIFPPSDEQLKSGTASVVCLLNNFYPREAKVQWKVDNALQSGNSQESVTEQDSKDSTYSLSSTLTLSKADYEKHKVYACEVTHQGLSSPVTKSFNRGEC

SEQ ID NO: 40 - DNA, 731 bp, Artificial Sequence
  Description of Artificial Sequence: Synthetic polypeptide
gctagcaccatgggctggagctgcatcatcctgttcctggtggccaccgccaccggcgtgcacagcgacatcgtgatgacccaggccgcccccagcgtggccgtgacccccggcgccagcgtgagcatcagctgccgcagcagcaagagcctgctgcacagcagcggcaagacctacctgtactggttcctgcagcgccccggccagagcccccagctgctgatctaccgcatgagcaacctggccagcggcgtgcccgaccgcttcagcggcagcggcagcggcaccgccttcaccctgcgcatcagccgcgtggaggccgaggacgtgggcgtgtactactgcatgcagcacctggagtacccctacaccttcggcggcggcaccaagctggagatcaagcgtacggtggccgctccttccgtgttcatcttccctccctccgacgagcagctgaagtccggcaccgcctccgtggtgtgtctgctgaacaacttctaccctcgggaggccaaggtgcagtggaaggtggacaacgccctgcagtccggcaactcccaggagtccgtcaccgagcaggactccaaggacagcacctactccctgtcctccaccctgaccctgtccaaggccgactacgagaagcacaaggtgtacgcctgtgaggtgacccaccagggcctgtccagccctgtgaccaagtccttcaaccggggcgagtgctgaagctt

SEQ ID NO: 41 - protein, 238 aa, Artificial Sequence
  Description of Artificial Sequence: Synthetic polypeptide
MGWSCIILFLVATATGVHSDIVMTQAAPSVAVTPGASVSISCRSSKSLLHSSGKTYLYWFLQRPGQSPQLLIYRLSNLASGVPDRFSGSGSGTAFTLRISRVEAEDVGVYYCMQHLEYPYTFGGGTKLEIKRTVAAPSVFIFPPSDEQLKSGTASVVCLLNNFYPREAKVQWKVDNALQSGNSQESVTEQDSKDSTYSLSSTLTLSKADYEKHKVYACEVTHQGLSSPVTKSFNRGEC

SEQ ID NO: 42 - DNA, 731 bp, Artificial Sequence
  Description of Artificial Sequence: Synthetic polynucleotide
gctagcaccatgggctggagctgcatcatcctgttcctggtggccaccgccaccggcgtgcacagcgacatcgtgatgacccaggccgcccccagcgtggccgtgacccccggcgccagcgtgagcatcagctgccgcagcagcaagagcctgctgcacagcagcggcaagacctacctgtactggttcctgcagcgccccggccagagcccccagctgctgatctaccgcctgagcaacctggccagcggcgtgcccgaccgcttcagcggcagcggcagcggcaccgccttcaccctgcgcatcagccgcgtggaggccgaggacgtgggcgtgtactactgcatgcagcacctggagtacccctacaccttcggcggcggcaccaagctggagatcaagcgtacggtggccgctccttccgtgttcatcttccctccctccgacgagcagctgaagtccggcaccgcctccgtggtgtgtctgctgaacaacttctaccctcgggaggccaaggtgcagtggaaggtggacaacgccctgcagtccggcaactcccaggagtccgtcaccgagcaggactccaaggacagcacctactccctgtcctccaccctgaccctgtccaaggccgactacgagaagcacaaggtgtacgcctgtgaggtgacccaccagggcctgtccagccctgtgaccaagtccttcaaccggggcgagtgctgaagctt

SEQ ID NO: 43 - protein, 238 aa, Artificial Sequence
  Description of Artificial Sequence: Synthetic polypeptide
MGWSCIILFLVATATGVHSDIVMTQAAPSVAVTPGASVSISCRSSKSLLHSSGKTYLYWFLQRPGQSPQLLIYRLSSLASGVPDRFSGSGSGTAFTLRISRVEAEDVGVYYCMQHLEYPYTFGGGTKLEIKRTVAAPSVFIFPPSDEQLKSGTASVVCLLNNFYPREAKVQWKVDNALQSGNSQESVTEQDSKDSTYSLSSTLTLSKADYEKHKVYACEVTHQGLSSPVTKSFNRGEC

SEQ ID NO: 44 - DNA, 731 bp, Artificial Sequence
  Description of Artificial Sequence: Synthetic polynucleotide
gctagcaccatgggctggagctgcatcatcctgttcctggtggccaccgccaccggcgtgcacagcgacatcgtgatgacccaggccgcccccagcgtggccgtgacccccggcgccagcgtgagcatcagctgccgcagcagcaagagcctgctgcacagcagcggcaagacctacctgtactggttcctgcagcgccccggccagagcccccagctgctgatctaccgcctgagcagcctggccagcggcgtgcccgaccgcttcagcggcagcggcagcggcaccgccttcaccctgcgcatcagccgcgtggaggccgaggacgtgggcgtgtactactgcatgcagcacctggagtacccctacaccttcggcggcggcaccaagctggagatcaagcgtacggtggccgctccttccgtgttcatcttccctccctccgacgagcagctgaagtccggcaccgcctccgtggtgtgtctgctgaacaacttctaccctcgggaggccaaggtgcagtggaaggtggacaacgccctgcagtccggcaactcccaggagtccgtcaccgagcaggactccaaggacagcacctactccctgtcctccaccctgaccctgtccaaggccgactacgagaagcacaaggtgtacgcctgtgaggtgacccaccagggcctgtccagccctgtgaccaagtccttcaaccggggcgagtgctgaagctt

SEQ ID NO: 45 - protein, 456 aa, Artificial Sequence
  Description of Artificial Sequence: Synthetic polypeptide
MGWSCIILFLVATATGVHSQVQLKESGPGLVAPSESLSITCTVSGFSLIDYGVNWIRQPPGKGLEWLGVIWGDGTTYYNPSLKSRLSISKDNSKSQVFLKVTSLTTDDTAMYYCARIVYWGQGTLVTVSAASTKGPSVFPLAPCSRSTSESTAALGCLVKDYFPEPVTVSWNSGALTSGVHTFPAVLQSSGLYSLSSVVTVPSSSLGTKTYTCNVDHKPSNTKVDKRVESKYGPPCPSCPAPEFLGGPSVFLFPPKPKDTLMISRTPEVTCVVVDVSQEDPEVQFNWYVDGVEVHNAKTKPREEQFNSTYRVVSVLTVLHQDWLNGKEYKCKVSNKGLPSSIEKTISKAKGQPREPQVYTLPPSQEEMTKNQVSLTCLVKGFYPSDIAVEWESNGQPENNYKTTPPVLDSDGSFFLYSRLTVDKSRWQEGNVFSCSVMHEALHNHYTQKSLSLSLG

SEQ ID NO: 46 - DNA, 1385 bp, Artificial Sequence
  Description of Artificial Sequence: Synthetic polynucleotide
gctagcaccatgggctggagctgcatcatcctgttcctggtggccaccgccaccggcgtgcacagccaggtgcagctgaaggagagcggccccggcctggtggcccccagcgagagcctgagcatcacctgcaccgtgagcggcttcagcctgatcgactacggcgtgaactggatccgccagccccccggcaagggcctggagtggctgggcgtgatctggggcgacggcaccacctactacaaccccagcctgaagagccgcctgagcatcagcaaggacaacagcaagagccaggtgttcctgaaggtgaccagcctgaccaccgacgacaccgccatgtactactgcgcccgcatcgtgtactggggccagggcaccctggtgaccgtgagcgccgccagcaccaagggcccttccgtgttccctctggccccttgctcccggtccacctccgagtccaccgccgctctgggctgcctggtgaaggactacttccctgagcctgtgaccgtgtcctggaactctggcgccctgacctccggcgtgcacaccttccctgccgtgctgcagtcctccggcctgtactccctgtcctccgtggtgaccgtgccttcctcctccctgggcaccaagacctacacctgtaacgtggaccacaagccttccaacaccaaggtggacaagcgggtggagtccaagtacggccctccttgcccttcctgccctgcccctgagttcctgggcggacctagcgtgttcctgttccctcctaagcctaaggacaccctgatgatctcccggacccctgaggtgacctgtgtggtggtggacgtgtcccaggaggaccctgaggtccagttcaactggtacgtggacggcgtggaggtgcacaacgccaagaccaagcctcgggaggagcagttcaattccacctaccgggtggtgtctgtgctgaccgtgctgcaccaggactggctgaacggcaaagaatacaagtgtaaggtctccaacaagggcctgccctcctccatcgagaaaaccatctccaaggccaagggccagcctagggagcctcaggtgtacaccctgcctcctagccaggaagagatgaccaagaaccaggtgtccctgacctgtctggtgaagggcttctacccttccgacatcgccgtggagtgggagtccaacggccagcctgagaacaactacaagaccacccctcctgtgctggactccgacggctccttcttcctgtactccaggctgaccgtggacaagtcccggtggcaggagggcaacgtcttttcctgctccgtgatgcacgaggccctgcacaaccactacacccagaagtccctgtccctgtctctgggctgaagctt

SEQ ID NO: 47 - protein, 456 aa, Artificial Sequence
  Description of Artificial Sequence: Synthetic polypeptide
MGWSCIILFLVATATGVHSEVQLKESGPGLVAPGGSLSITCTVSGFSLIDYGVNWIRQPPGKGLEWLGVIWGDGTTYYNAPLKGRLSISKDNSKSQVFLQMNSLKTDDTAMYYCARIVYWGQGTLVTVSSASTKGPSVFPLAPCSRSTSESTAALGCLVKDYFPEPVTVSWNSGALTSGVHTFPAVLQSSGLYSLSSVVTVPSSSLGTKTYTCNVDHKPSNTKVDKRVESKYGPPCPSCPAPEFLGGPSVFLFPPKPKDTLMISRTPEVTCVVVDVSQEDPEVQFNWYVDGVEVHNAKTKPREEQFNSTYRVVSVLTVLHQDWLNGKEYKCKVSNKGLPSSIEKTISKAKGQPREPQVYTLPPSQEEMTKNQVSLTCLVKGFYPSDIAVEWESNGQPENNYKTTPPVLDSDGSFFLYSRLTVDKSRWQEGNVFSCSVMHEALHNHYTQKSLSLSLG

SEQ ID NO: 48 - DNA, 1385 bp, Artificial Sequence
  Description of Artificial Sequence: Synthetic polynucleotide
gctagcaccatgggctggagctgcatcatcctgttcctggtggccaccgccaccggcgtgcacagcgaggtgcagctgaaggagagcggccccggcctggtggcccccggcggcagcctgagcatcacctgcaccgtgagcggcttcagcctgatcgactacggcgtgaactggatccgccagccccccggcaagggcctggagtggctgggcgtgatctggggcgacggcaccacctactacaacgcccccctgaagggccgcctgagcatcagcaaggacaacagcaagagccaggtgttcctgcagatgaacagcctgaagaccgacgacaccgccatgtactactgcgcccgcatcgtgtactggggccagggcaccctggtgaccgtgagcagcgccagcaccaagggcccttccgtgttccctctggccccttgctcccggtccacctccgagtccaccgccgctctgggctgcctggtgaaggactacttccctgagcctgtgaccgtgtcctggaactctggcgccctgacctccggcgtgcacaccttccctgccgtgctgcagtcctccggcctgtactccctgtcctccgtggtgaccgtgccttcctcctccctgggcaccaagacctacacctgtaacgtggaccacaagccttccaacaccaaggtggacaagcgggtggagtccaagtacggccctccttgcccttcctgccctgcccctgagttcctgggcggacctagcgtgttcctgttccctcctaagcctaaggacaccctgatgatctcccggacccctgaggtgacctgtgtggtggtggacgtgtcccaggaggaccctgaggtccagttcaactggtacgtggacggcgtggaggtgcacaacgccaagaccaagcctcgggaggagcagttcaattccacctaccgggtggtgtctgtgctgaccgtgctgcaccaggactggctgaacggcaaagaatacaagtgtaaggtctccaacaagggcctgccctcctccatcgagaaaaccatctccaaggccaagggccagcctagggagcctcaggtgtacaccctgcctcctagccaggaagagatgaccaagaaccaggtgtccctgacctgtctggtgaagggcttctacccttccgacatcgccgtggagtgggagtccaacggccagcctgagaacaactacaagaccacccctcctgtgctggactccgacggctccttcttcctgtactccaggctgaccgtggacaagtcccggtggcaggagggcaacgtcttttcctgctccgtgatgcacgaggccctgcacaaccactacacccagaagtccctgtccctgtctctgggctgaagctt

SEQ ID NO: 49 - protein, 5 aa, Homo sapiens
ELLGG

SEQ ID NO: 50 - protein, 5 aa, Homo sapiens
MISRT

SEQ ID NO: 51 - protein, 6 aa, Artificial Sequence
  Description of Artificial Sequence: Synthetic 6x His tag
HHHHHH

SEQ ID NO: 52 - protein, 15 aa, Artificial Sequence
  Description of Artificial Sequence: Synthetic peptide
PGKAPQLLIYRMSNL

SEQ ID NO: 53 - protein, 15 aa, Artificial Sequence
  Description of Artificial Sequence: Synthetic peptide
PGKAPKLLIYAASSL

SEQ ID NO: 54 - protein, 15 aa, Artificial Sequence
  Description of Artificial Sequence: Synthetic peptide
SLIDYGVNWIRQPPG

SEQ ID NO: 55 - protein, 112 aa, Artificial Sequence
  Description of Artificial Sequence: Synthetic polypeptide
DIVMTQAAPSVAVTPGQSVSISCRSSKSLLHSSGKTYLYWFLQHPGKAPQLLIYRMSNLASGVPDRFSGSGSGTAFTLTISGVQAEDVGVYYCMQHLEYPYTFGGGTKLEIK

SEQ ID NO: 56 - protein, 113 aa, Artificial Sequence
  Description of Artificial Sequence: Synthetic polypeptide
QVQLQESGPGLVAPSQSLSITCTVSGFSLIDYGVNWIRQPPGKGLEWLGVIWGDGTTYYNSALKSRLSISKDTSKSQVFLKMNSLTTDDTAMYYCARIVYWGQGTLVTVSAAK

SEQ ID NO: 57 - protein, 113 aa, Artificial Sequence
  Description of Artificial Sequence: Synthetic polypeptide
QVQLQESGPGLVAPSQSLSITCTVSGFSLIDYGVNWIRQPPGKGLEWLGVIWGDGTTYYPSALKSRLSISKDTSKSQVFLKMNSLTTDDTAMYYCARIVYWGQGTLVTVSAAK

SEQ ID NO: 58 - protein, 16 aa, Artificial Sequence
  Synthetic peptide
RSSKSLLHSSGKTYLY

SEQ ID NO: 59 - protein, 7 aa, Artificial Sequence
  Synthetic peptide
RMSNLAS

SEQ ID NO: 60 - protein, 9 aa, Artificial Sequence
  Synthetic peptide
MQHLEYPYT

SEQ ID NO: 61 - protein, 10 aa, Artificial Sequence
  Synthetic peptide
GFSLIDYGVN

SEQ ID NO: 62 - protein, 9 aa, Artificial Sequence
  Synthetic peptide
VIWGDGTTY

SEQ ID NO: 63 - protein, 3 aa, Artificial Sequence
  Synthetic peptide
IVY

SEQ ID NO: 64 - protein, 7 aa, Artificial Sequence
  Synthetic peptide
RLSNLAS

SEQ ID NO: 65 - protein, 8 aa, Artificial Sequence
  Synthetic peptide
RLSSNLAS

SEQ ID NO: 66 - protein, 6 aa, Artificial Sequence
  Synthetic peptide
RMSNLA

SEQ ID NO: 67 - protein, 6 aa, Artificial Sequence
  Synthetic peptide
RLSNLA

SEQ ID NO: 68 - protein, 6 aa, Artificial Sequence
  Synthetic peptide
RLSSLA

SEQ ID NO: 69 - protein, 17 aa, Artificial Sequence
  Synthetic peptide
RSSKSLLHSSGKTYLYW